European Patent Application EP 4 682 174 A1, published January 21, 2026. Title: UNIVERSAL INFLUENZA MRNA VACCINE AND USE THEREOF. Applicant: SHANGHAI INSTITUTE OF BIOLOGICAL PRODUCTS CO., LTD. The sequence listing filed with the application follows.

SEQUENCE LISTING (14 sequences)

SEQ ID NO: 1 - protein, 791 aa, synthetic construct
  source 1..791: note = M2e-LAH-NP Protein
MDAMKRGLCCVLLLCGAVFVSPSSLLTEVETPIRNEWGSRSNGGSLLTEVETPTRSEWESRSSGGSLLTEVETPTRNEWESRSSGGSLLTEVETLTRNGWGCRCSGGRMENLNKKVDDGFLDIWTYNAELLVLLENERTLDFHDSNVKNLYEKVKSQLKNNAGGSRIQDLEKYVEDTKIDLWSYNAELLVALENQHTIDLTDSEMNKLFEKTRRQLRENAGGSRIENLNKKMEDGFLDVWTYNAELLVLMENERTLDFHDSNVKNLYDKVRLQLRDNAGGGSGGGSGGGSGGGSASQGTPPSYEQMETDGERQNATEIRASVGKMIGGIGRFYIQMCTELKLSDYEGRLIQNSLTIERMVLSAFDERRNKYLEEHPSAGKDPKKTGGPIYRRVNGKWMRELILYDKEEIRRIWRQANNGDDATAGLTHMMIWHSNLNDATYQRTRALVRTGMDPRMCSLMQGSTLPRRSGAAGAAVKGVGTMVMELVRMIKRGINDRNFWRGENGPPTPIAYERMCNILKGKFQTAAQKAMMDQVRESRNPGNAEFEDLTFLARSALILRGSVAHKSCLPACVYGPAVASGYDFEREGYSLVGIDPFRLLQNSQVYSLIRPNENPAHKSQLVWMACHSAAFEDLPLLSFIKGTKVVPRGKLSTRGVQIASNENMETMESSTLELRSRYWAIRTRSGGNTNQQRASAGQISIQPTFSVQRNLPFDRTTIMAAFTGNTEGRTSDMRTEIIRMMESARPEDVSFQGRGVFELSDEKAASPIVPSFDMSNEGSYFFGDNAEEYDN

SEQ ID NO: 2 - RNA, 2376 nt, synthetic construct
  source 1..2376: mol_type = other RNA; note = mRNA vaccine
atggacgccatgaagagaggcctctgctgcgtgctgctgctgtgcggcgccgtgttcgtgagccccagctccctcctcacagaggtggagacacccatccggaacgagtggggcagcagaagcaacggaggcagcctcctcaccgaggtggagacacccaccagatccgagtgggagagcagatccagcggaggcagcctcctgaccgaggtggagacacccaccagaaacgagtgggagagcagatccagcggaggcagcctcctgaccgaggtggagacactcaccagaaacggctggggctgcagatgcagcggcggacggatggagaacttaaacaagaaggtggacgacggcttcctggacatctggacctacaacgccgagttgttagtgctactggagaacgagcggaccctggacttccacgacagcaacgtgaagaacctgtacgagaaggtgaagtcccagttaaagaacaacgctggaggcagccggatccaggacctggagaagtacgtggaggacaccaagatcgacctttggagctacaacgccgagcttctcgtggctctggagaaccagcacaccatcgacctcaccgacagcgagatgaacaagttgttcgagaagaccagacggcagctgcgggagaacgctggaggcagccggatcgagaacttgaacaagaagatggaggacggcttcctcgacgtgtggacctacaacgccgagttgttggtgctcatggagaacgagagaaccctcgacttccacgactccaacgtgaagaacctttacgacaaggtgcggttacagctgagagacaacgctggcggaggcagcggcggaggctccggcggaggcagcggcggaggctccgccagccagggcacccctcccagctacgagcagatggagacagacggcgagcggcagaacgccaccgagatcagagccagcgtgggcaagatgatcggcggcatcggccggttctacatccagatgtgcaccgagctgaagctcagcgactacgagggcagattgatccagaacagcttaaccatcgagcggatggtgctcagcgccttcgacgagagacggaacaagtacctggaggagcaccccagcgccggcaaggaccccaagaagaccggcggccctatctaccggagagtgaacggcaagtggatgcgggagctcatcctttacgacaaggaggagatcagacggatctggcggcaggccaacaacggcgacgacgccaccgctggcctgacccacatgatgatctggcacagcaacttgaacgacgccacctaccagcggaccagagcccttgtgcggaccggcatggaccctcggatgtgcagcctgatgcagggcagcaccctccctagacggtccggcgctgccggcgctgccgtgaagggcgtgggcaccatggtgatggagttggtgcggatgatcaagagaggcatcaacgaccggaacttctggagaggcgagaacggccctcccacacccatcgcctacgagcggatgtgcaacatcctcaagggcaagttccagacagccgcccagaaggccatgatggaccaggtgcgggagagccggaaccctggcaacgccgagttcgaggacctcaccttcctagcccggagcgccctcatcttgcggggcagcgtggcccacaagagctgcctgcctgcctgcgtgtacggccctgccgtggccagcggctacgacttcgagcgggagggctacagcctagtgggcatcgaccccttccggctgcttcagaacagccaggtgtactccctaatcagacccaacgagaaccccgcccacaagtcccagctggtgtggatggcctgccacagcgccgccttcgaggacctacccttattaagcttcatcaagggcaccaaggtggtgcctcggggcaagcttagcacacggggcgtgcagatcgccagcaacgagaacatggagacaatggagtccagcacccttgagctgcggagccggtactgggccatccggaccagaagcggcggcaacaccaaccagcagagagccagcgctggccagatcagcatccagcccaccttcagcgtgcagcggaacctccccttcgaccggaccaccatcatggccgccttcacaggcaacaccgagggcagaacctccgacatgcggaccgagatcatccggatgatggagagcgcaagaccagaggacgtgagcttccagggcagaggcgtgttcgagctcagcgacgagaaggccgccagccccatcgtgcccagcttcgacatgagcaacgagggcagctacttcttcggcgacaacgccgaggagtacgacaactga

SEQ ID NO: 3 - protein, 19 aa, synthetic construct
  source 1..19: note = M2e
SLLTEVETPIRNEWGSRSN

SEQ ID NO: 4 - protein, 19 aa, synthetic construct
  source 1..19: note = M2e
SLLTEVETPTRSEWESRSS

SEQ ID NO: 5 - protein, 19 aa, synthetic construct
  source 1..19: note = M2e
SLLTEVETPTRNEWESRSS

SEQ ID NO: 6 - protein, 19 aa, synthetic construct
  source 1..19: note = M2e
SLLTEVETLTRNGWGCRCS

SEQ ID NO: 7 - protein, 55 aa, synthetic construct
  source 1..55: note = LAH
RMENLNKKVDDGFLDIWTYNAELLVLLENERTLDFHDSNVKNLYEKVKSQLKNNA

SEQ ID NO: 8 - protein, 55 aa, synthetic construct
  source 1..55: note = LAH
RIQDLEKYVEDTKIDLWSYNAELLVALENQHTIDLTDSEMNKLFEKTRRQLRENA

SEQ ID NO: 9 - protein, 55 aa, synthetic construct
  source 1..55: note = LAH
RIENLNKKMEDGFLDVWTYNAELLVLMENERTLDFHDSNVKNLYDKVRLQLRDNA

SEQ ID NO: 10 - protein, 497 aa, synthetic construct
  source 1..497: note = mutated NP
ASQGTPPSYEQMETDGERQNATEIRASVGKMIGGIGRFYIQMCTELKLSDYEGRLIQNSLTIERMVLSAFDERRNKYLEEHPSAGKDPKKTGGPIYRRVNGKWMRELILYDKEEIRRIWRQANNGDDATAGLTHMMIWHSNLNDATYQRTRALVRTGMDPRMCSLMQGSTLPRRSGAAGAAVKGVGTMVMELVRMIKRGINDRNFWRGENGPPTPIAYERMCNILKGKFQTAAQKAMMDQVRESRNPGNAEFEDLTFLARSALILRGSVAHKSCLPACVYGPAVASGYDFEREGYSLVGIDPFRLLQNSQVYSLIRPNENPAHKSQLVWMACHSAAFEDLPLLSFIKGTKVVPRGKLSTRGVQIASNENMETMESSTLELRSRYWAIRTRSGGNTNQQRASAGQISIQPTFSVQRNLPFDRTTIMAAFTGNTEGRTSDMRTEIIRMMESARPEDVSFQGRGVFELSDEKAASPIVPSFDMSNEGSYFFGDNAEEYDN

SEQ ID NO: 11 - protein, 23 aa, synthetic construct
  source 1..23: note = Signal peptide
MDAMKRGLCCVLLLCGAVFVSPS

SEQ ID NO: 12 - protein, 82 aa, synthetic construct
  source 1..82: note = M2e
SLLTEVETPIRNEWGSRSNGGSLLTEVETPTRSEWESRSSGGSLLTEVETPTRNEWESRSSGGSLLTEVETLTRNGWGCRCS

SEQ ID NO: 13 - protein, 171 aa, synthetic construct
  source 1..171: note = LAH
RMENLNKKVDDGFLDIWTYNAELLVLLENERTLDFHDSNVKNLYEKVKSQLKNNAGGSRIQDLEKYVEDTKIDLWSYNAELLVALENQHTIDLTDSEMNKLFEKTRRQLRENAGGSRIENLNKKMEDGFLDVWTYNAELLVLMENERTLDFHDSNVKNLYDKVRLQLRDNA

SEQ ID NO: 14 - protein, 16 aa, synthetic construct
  source 1..16: note = linker
GGGSGGGSGGGSGGGS